European Patent Specification EP 4 125 985 B1, published January 7, 2026. Title: Methods for producing heme peroxidases. Applicant: TECHNISCHE UNIVERSITÄT WIEN. The sequence listing filed with the application follows.

SEQUENCE LISTING (8 sequences)

SEQ ID NO: 1 - protein, 306 aa, Armoracia rusticana
QLTPTFYDNSCPNVSNIVRDTIVNELRSDPRIAASILRLHFHDCFVNGCDASILLDNTTSFRTEKDAFGNANSARGFPVIDRMKAAVESACPRTVSCADLLTIAAQQSVTLAGGPSWRVPLGRRDSLQAFLDLANANLPAPFFTLPQLKDSFRNVGLNRSSDLVALSGGHTFGKNQCRFIMDRLYNFSNTGLPDPTLNTTYLQTLRGLCPLNGNLSALVDFDLRTPTIFDNKYYVNLEEQKGLIQSDQELFSSPNATDTIPLVRSFANSTQTFFNAFVEAMDRMGNITPLTGTQGQIRLNCRVVNS

SEQ ID NO: 2 - protein, 307 aa, Artificial Sequence
  recombinant wt HRP
MQLTPTFYDNSCPNVSNIVRDTIVNELRSDPRIAASILRLHFHDCFVNGCDASILLDNTTSFRTEKDAFGNANSARGFPVIDRMKAAVESACPRTVSCADLLTIAAQQSVTLAGGPSWRVPLGRRDSLQAFLDLANANLPAPFFTLPQLKDSFRNVGLNRSSDLVALSGGHTFGKNQCRFIMDRLYNFSNTGLPDPTLNTTYLQTLRGLCPLNGNLSALVDFDLRTPTIFDNKYYVNLEEQKGLIQSDQELFSSPNATDTIPLVRSFANSTQTFFNAFVEAMDRMGNITPLTGTQGQIRLNCRVVNS

SEQ ID NO: 3 - protein, 306 aa, Artificial Sequence
  HRP N13D/N57S/P146Q/N175S/N255D/N268D/N275K
QLTPTFYDNSCPDVSNIVRDTIVNELRSDPRIAASILRLHFHDCFVNGCDASILLDSTTSFRTEKDAFGNANSARGFPVIDRMKAAVESACPRTVSCADLLTIAAQQSVTLAGGPSWRVPLGRRDSLQAFLDLANANLPAPFFTLQQLKDSFRNVGLNRSSDLVALSGGHTFGKSQCRFIMDRLYNFSNTGLPDPTLNTTYLQTLRGLCPLNGNLSALVDFDLRTPTIFDNKYYVNLEEQKGLIQSDQELFSSPDATDTIPLVRSFADSTQTFFKAFVEAMDRMGNITPLTGTQGQIRLNCRVVNS

SEQ ID NO: 4 - protein, 307 aa, Artificial Sequence
  recombinant HRP N13D/N57S/P146Q/N175S/N255D/N268D/N275K
MQLTPTFYDNSCPDVSNIVRDTIVNELRSDPRIAASILRLHFHDCFVNGCDASILLDSTTSFRTEKDAFGNANSARGFPVIDRMKAAVESACPRTVSCADLLTIAAQQSVTLAGGPSWRVPLGRRDSLQAFLDLANANLPAPFFTLQQLKDSFRNVGLNRSSDLVALSGGHTFGKSQCRFIMDRLYNFSNTGLPDPTLNTTYLQTLRGLCPLNGNLSALVDFDLRTPTIFDNKYYVNLEEQKGLIQSDQELFSSPDATDTIPLVRSFADSTQTFFKAFVEAMDRMGNITPLTGTQGQIRLNCRVVNS

SEQ ID NO: 5 - DNA, 28 bp, Artificial Sequence
  DHU_P146deg3_fwd
  misc_difference 11: /note="a or g or c or t"
  misc_difference 12: /note="a or g or c or t"
tttcacgctgnnkcaactgaaagatagc

SEQ ID NO: 6 - DNA, 24 bp, Artificial Sequence
  DHU_P146deg3_rev
aacggagccggcagattagcgttt

SEQ ID NO: 7 - DNA, 27 bp, Artificial Sequence
  DHU_N275deg3_fwd
  misc_difference 11: /note="a or g or c or t"
  misc_difference 12: /note="a or g or c or t"
gacgtttttcnnkgcattcgtcgaagc

SEQ ID NO: 8 - DNA, 23 bp, Artificial Sequence
  DHU_N275deg3_rev
tgggtcgaatcggcaaatgaacg